European Patent Specification EP 4 060 031 B1, published November 5, 2025. Title: Novel 3-deoxy-D-arabinoheptulosonate-7-phosphate synthase variant and a method for producing L-lysine using the same. Applicant: CJ CheilJedang Corporation. The sequence listing filed with the application follows.

SEQUENCE LISTING (10 sequences)

SEQ ID NO: 1 - protein, 466 aa, Artificial Sequence
  (G382C)_3-deoxy-D-arabinoheptulosonate-7-phosphate synthase
MNRGVSWTVDIPKEVLPDLPPLPEGMQQQFEDTISRDAKQQPTWDRAQAENVRKILESVPPIVVAPEVLELKQKLADVANGKAFLLQGGDCAETFESNTEPHIRANVKTLLQMAVVLTYGASTPVIKMARIAGQYAKPRSSDLDGNGLPNYRGDIVNGVEATPEARRHDPARMIRAYANASAAMNLVRALTSSGTADLYRLSEWNREFVANSPAGARYEALAREIDSGLRFMEACGVSDESLRAADIYCSHEALLVDYERSMLRLATDEEGNEELYDLSAHQLWIGERTRGMDDFHVNFASMISNPIGIKIGPGITPEEAVAYADKLDPNFEPGRLTIVARMGHDKVRSVLPGVIQAVEASGHKVIWQSDPMHGNTFTASNCYKTRHFDKVIDEVQGFFEVHRALGTHPGGIHIEFTGEDVTECLGGAEDITDVDLPGRYESACDPRLNTQQSLELAFLVAEMLRN

SEQ ID NO: 2 - DNA, 1401 bp, Artificial Sequence
  (G382C)_NCgl2098
atgaataggggtgtgagttggacagttgatatccctaaagaagttctccctgatttgccaccattgccagaaggcatgcagcagcagttcgaggacaccatttcccgtgacgctaagcagcaacctacgtgggatcgtgcacaggcagaaaacgtgcgcaagatccttgagtcggttcctccaatcgttgttgcccctgaggtacttgagctgaagcagaagcttgctgatgttgccaacggtaaggccttcctcttgcagggtggtgactgtgcggaaactttcgagtcaaacactgagccgcacattcgcgccaacgtaaagactctgctgcagatggcagttgttttgacctacggtgcatccactcctgtgatcaagatggctcgtattgctggtcagtacgcaaagcctcgctcttctgatctggatggaaatggtctgccaaactaccgtggcgatatcgtcaacggtgtggaggcaaccccagaggctcgtcgccacgatcctgcccgcatgatccgtgcttacgctaacgcttctgctgcgatgaacttggtgcgcgcgctcaccagctctggcaccgctgatctttaccgtctcagcgagtggaaccgcgagttcgttgcgaactccccagctggtgcacgctacgaggctcttgctcgtgagatcgactccggtctgcgcttcatggaagcatgtggcgtgtccgatgagtccctgcgtgctgcagatatctactgctcccacgaggctttgctggtggattacgagcgttccatgctgcgtcttgcaaccgatgaggaaggcaacgaggaactttacgatctttcagctcaccagctgtggatcggcgagcgcacccgtggcatggatgatttccatgtgaacttcgcatccatgatctctaacccaatcggcatcaagattggtcctggtatcacccctgaagaggctgttgcatacgctgacaagctcgatccgaacttcgagcctggccgtttgaccatcgttgctcgcatgggccacgacaaggttcgctccgtacttcctggtgttatccaggctgttgaggcatccggacacaaggttatttggcagtccgatccgatgcacggcaacactttcaccgcatccaattgctacaagacccgtcacttcgacaaggttatcgatgaggtccagggcttcttcgaggtccaccgcgcattgggcacccacccaggcggaatccacattgagttcactggtgaagatgtcaccgagtgcctcggtggcgctgaagacatcaccgatgttgatctgccaggccgctacgagtccgcatgcgatcctcgcctgaacactcagcagtctttggagttggctttcctcgttgcagaaatgctgcgtaactaa

SEQ ID NO: 3 - protein, 466 aa, Artificial Sequence
  (WT)_3-deoxy-D-arabinoheptulosonate-7-phosphate synthase
MNRGVSWTVDIPKEVLPDLPPLPEGMQQQFEDTISRDAKQQPTWDRAQAENVRKILESVPPIVVAPEVLELKQKLADVANGKAFLLQGGDCAETFESNTEPHIRANVKTLLQMAVVLTYGASTPVIKMARIAGQYAKPRSSDLDGNGLPNYRGDIVNGVEATPEARRHDPARMIRAYANASAAMNLVRALTSSGTADLYRLSEWNREFVANSPAGARYEALAREIDSGLRFMEACGVSDESLRAADIYCSHEALLVDYERSMLRLATDEEGNEELYDLSAHQLWIGERTRGMDDFHVNFASMISNPIGIKIGPGITPEEAVAYADKLDPNFEPGRLTIVARMGHDKVRSVLPGVIQAVEASGHKVIWQSDPMHGNTFTASNGYKTRHFDKVIDEVQGFFEVHRALGTHPGGIHIEFTGEDVTECLGGAEDITDVDLPGRYESACDPRLNTQQSLELAFLVAEMLRN

SEQ ID NO: 4 - DNA, 1401 bp, Artificial Sequence
  (WT)_NCgl2098
atgaataggggtgtgagttggacagttgatatccctaaagaagttctccctgatttgccaccattgccagaaggcatgcagcagcagttcgaggacaccatttcccgtgacgctaagcagcaacctacgtgggatcgtgcacaggcagaaaacgtgcgcaagatccttgagtcggttcctccaatcgttgttgcccctgaggtacttgagctgaagcagaagcttgctgatgttgccaacggtaaggccttcctcttgcagggtggtgactgtgcggaaactttcgagtcaaacactgagccgcacattcgcgccaacgtaaagactctgctgcagatggcagttgttttgacctacggtgcatccactcctgtgatcaagatggctcgtattgctggtcagtacgcaaagcctcgctcttctgatctggatggaaatggtctgccaaactaccgtggcgatatcgtcaacggtgtggaggcaaccccagaggctcgtcgccacgatcctgcccgcatgatccgtgcttacgctaacgcttctgctgcgatgaacttggtgcgcgcgctcaccagctctggcaccgctgatctttaccgtctcagcgagtggaaccgcgagttcgttgcgaactccccagctggtgcacgctacgaggctcttgctcgtgagatcgactccggtctgcgcttcatggaagcatgtggcgtgtccgatgagtccctgcgtgctgcagatatctactgctcccacgaggctttgctggtggattacgagcgttccatgctgcgtcttgcaaccgatgaggaaggcaacgaggaactttacgatctttcagctcaccagctgtggatcggcgagcgcacccgtggcatggatgatttccatgtgaacttcgcatccatgatctctaacccaatcggcatcaagattggtcctggtatcacccctgaagaggctgttgcatacgctgacaagctcgatccgaacttcgagcctggccgtttgaccatcgttgctcgcatgggccacgacaaggttcgctccgtacttcctggtgttatccaggctgttgaggcatccggacacaaggttatttggcagtccgatccgatgcacggcaacactttcaccgcatccaatggctacaagacccgtcacttcgacaaggttatcgatgaggtccagggcttcttcgaggtccaccgcgcattgggcacccacccaggcggaatccacattgagttcactggtgaagatgtcaccgagtgcctcggtggcgctgaagacatcaccgatgttgatctgccaggccgctacgagtccgcatgcgatcctcgcctgaacactcagcagtctttggagttggctttcctcgttgcagaaatgctgcgtaactaa

SEQ ID NO: 5 - DNA, 40 bp, Artificial Sequence
  NCgl2098_1F
tgaattcgagctcggtacccttcgttgcgaactccccagc

SEQ ID NO: 6 - DNA, 33 bp, Artificial Sequence
  NCgl2098_2R
tgacgggtcttgtagcaattggatgcggtgaaa

SEQ ID NO: 7 - DNA, 33 bp, Artificial Sequence
  NCgl2098_3F
tttcaccgcatccaattgctacaagacccgtca

SEQ ID NO: 8 - DNA, 40 bp, Artificial Sequence
  NCgl2098_4R
gtcgactctagaggatccccagttatcttgagcgtcatgc

SEQ ID NO: 9 - DNA, 20 bp, Artificial Sequence
  NCgl2098_5F
ttcgttgcgaactccccagc

SEQ ID NO: 10 - DNA, 20 bp, Artificial Sequence
  NCgl2098_6R
agttatcttgagcgtcatgc